European Patent Specification EP 3 995 591 B1, published January 10, 2024. Title: NUCLEASE PROFILING SYSTEM. Applicant: President and Fellows of Harvard College. The sequence listing filed with the application follows.

SEQUENCE LISTING (410 sequences)

SEQ ID NO: 1 - DNA, 23 bp, Artificial Sequence
  Synthetic Polynucleotide
  misc_feature (21)..(21): n is a, c, g, or t
agtcctcatctccctcaagcngg

SEQ ID NO: 2 - DNA, 48 bp, Artificial Sequence
  Synthetic Oligonucleotide
atgtctcccgcatgcgctcagtcctcatctccctcaagcaggccccgc

SEQ ID NO: 3 - DNA, 48 bp, Artificial Sequence
  Synthetic Oligonucleotide
gcggggcctgcttgagggagatgaggactgagcgcatgcgggagacat

SEQ ID NO: 4 - DNA, 48 bp, Artificial Sequence
  Synthetic Oligonucleotide
tggtgcactgaagagccaccctgtggaaacactacatctgcaatatct

SEQ ID NO: 5 - DNA, 48 bp, Artificial Sequence
  Synthetic Oligonucleotide
agatattgcagatgtagtgtttccacagggtggctcttcagtgcacca

SEQ ID NO: 6 - DNA, 48 bp, Artificial Sequence
  Synthetic Oligonucleotide
taatcctactcagtgaagctcttcacagtcattggattaattatgttg

SEQ ID NO: 7 - DNA, 48 bp, Artificial Sequence
  Synthetic Oligonucleotide
caacataattaatccaatgactgtgaagagcttcactgagtaggatta

SEQ ID NO: 8 - DNA, 23 bp, Artificial Sequence
  Synthetic Oligonucleotide
agtcctcatctccctcaagcagg

SEQ ID NO: 9 - DNA, 23 bp, Artificial Sequence
  Synthetic Oligonucleotide
cctgcttgagggagatgaggact

SEQ ID NO: 10 - RNA, 60 nt, Artificial Sequence
  Synthetic Oligonucleotide
gaguccucaucucccucaagcguuuuagagcuagaaauagcuuaaaauaaggcuaguccg

SEQ ID NO: 11 - DNA, 23 bp, Artificial Sequence
  Synthetic Oligonucleotide
ctccctcaagcaggccccgctgg

SEQ ID NO: 12 - DNA, 23 bp, Artificial Sequence
  Synthetic Oligonucleotide
ccagcggggcctgcttgagggag

SEQ ID NO: 13 - RNA, 60 nt, Artificial Sequence
  Synthetic Oligonucleotide
gcucccucaagcaggccccgcguuuuagagcuagaaauagcuuaaaauaaggcuaguccg

SEQ ID NO: 14 - DNA, 23 bp, Artificial Sequence
  Synthetic Oligonucleotide
tgtgaagagcttcactgagtagg

SEQ ID NO: 15 - DNA, 23 bp, Artificial Sequence
  Synthetic Oligonucleotide
cctactcagtgaagctcttcaca

SEQ ID NO: 16 - RNA, 60 nt, Artificial Sequence
  Synthetic Oligonucleotide
gugugaagagcuucacugaguguuuuagagcuagaaauagcuuaaaauaaggcuaguccg

SEQ ID NO: 17 - DNA, 23 bp, Artificial Sequence
  Synthetic Oligonucleotide
gcagatgtagtgtttccacaggg

SEQ ID NO: 18 - DNA, 23 bp, Artificial Sequence
  Synthetic Oligonucleotide
ccctgtggaaacactacatctgc

SEQ ID NO: 19 - RNA, 60 nt, Artificial Sequence
  Synthetic Oligonucleotide
ggcagauguaguguuuccacaguuuuagagcuagaaauagcuuaaaauaaggcuaguccg

SEQ ID NO: 20 - DNA, 23 bp, Artificial Sequence
  Synthetic Oligonucleotide
agtcctcatctccctcaagcagg

SEQ ID NO: 21 - DNA, 23 bp, Artificial Sequence
  Synthetic Oligonucleotide
cctgcttgagggagatgaggact

SEQ ID NO: 22 - RNA, 73 nt, Artificial Sequence
  Synthetic Oligonucleotide
gaguccucaucucccucaagcguuuuagagcuaugcugaaaagcauagcuuaaaauaaggcuaguccguuauc

SEQ ID NO: 23 - DNA, 23 bp, Artificial Sequence
  Synthetic Oligonucleotide
ctccctcaagcaggccccgctgg

SEQ ID NO: 24 - DNA, 23 bp, Artificial Sequence
  Synthetic Oligonucleotide
ccagcggggcctgcttgagggag

SEQ ID NO: 25 - RNA, 73 nt, Artificial Sequence
  Synthetic Oligonucleotide
gcucccucaagcaggccccgcguuuuagagcuaugcugaaaagcauagcuuaaaauaaggcuaguccguuauc

SEQ ID NO: 26 - DNA, 23 bp, Artificial Sequence
  Synthetic Oligonucleotide
tgtgaagagcttcactgagtagg

SEQ ID NO: 27 - DNA, 23 bp, Artificial Sequence
  Synthetic Oligonucleotide
cctactcagtgaagctcttcaca

SEQ ID NO: 28 - RNA, 73 nt, Artificial Sequence
  Synthetic Oligonucleotide
gugugaagagcuucacugaguguuuuagagcuaugcugaaaagcauagcuuaaaauaaggcuaguccguuauc

SEQ ID NO: 29 - DNA, 23 bp, Artificial Sequence
  Synthetic Oligonucleotide
gcagatgtagtgtttccacaggg

SEQ ID NO: 30 - DNA, 23 bp, Artificial Sequence
  Synthetic Oligonucleotide
ccctgtggaaacactacatctgc

SEQ ID NO: 31 - RNA, 73 nt, Artificial Sequence
  Synthetic Oligonucleotide
ggcagauguaguguuuccacaguuuuagagcuaugcugaaaagcauagcuuaaaauaaggcuaguccguuauc

SEQ ID NO: 32 - DNA, 23 bp, Artificial Sequence
  Synthetic Oligonucleotide
  misc_feature (21)..(21): n is a, c, g, or t
ctccctcaagcaggccccgcngg

SEQ ID NO: 33 - DNA, 23 bp, Artificial Sequence
  Synthetic Oligonucleotide
  misc_feature (21)..(21): n is a, c, g, or t
gcagatgtagtgtttccacangg

SEQ ID NO: 34 - DNA, 23 bp, Artificial Sequence
  Synthetic Oligonucleotide
gcagatgtagtgtttccacaggg

SEQ ID NO: 35 - DNA, 23 bp, Artificial Sequence
  Synthetic Oligonucleotide
gaagatgtagtgtttccacaggg

SEQ ID NO: 36 - DNA, 23 bp, Artificial Sequence
  Synthetic Oligonucleotide
gaagatgtagtgtttccactggg

SEQ ID NO: 37 - DNA, 23 bp, Artificial Sequence
  Synthetic Oligonucleotide
gcagatggagggtttccacaggg

SEQ ID NO: 38 - DNA, 23 bp, Artificial Sequence
  Synthetic Oligonucleotide
gcagatgtagtgttaccagaggg

SEQ ID NO: 39 - DNA, 23 bp, Artificial Sequence
  Synthetic Oligonucleotide
ggggatgtagtgtttccactggg

SEQ ID NO: 40 - DNA, 4104 bp, Artificial Sequence
  Synthetic Oligonucleotide
atggataagaaatactcaataggcttagatatcggcacaaatagcgtcggatgggcggtgatcactgatgattataaggttccgtctaaaaagttcaaggttctgggaaatacagaccgccacagtatcaaaaaaaatcttataggggctcttttatttggcagtggagagacagcggaagcgactcgtctcaaacggacagctcgtagaaggtatacacgtcggaagaatcgtatttgttatctacaggagattttttcaaatgagatggcgaaagtagatgatagtttctttcatcgacttgaagagtcttttttggtggaagaagacaagaagcatgaacgtcatcctatttttggaaatatagtagatgaagttgcttatcatgagaaatatccaactatctatcatctgcgaaaaaaattggcagattctactgataaagcggatttgcgcttaatctatttggccttagcgcatatgattaagtttcgtggtcattttttgattgagggagatttaaatcctgataatagtgatgtggacaaactatttatccagttggtacaaatctacaatcaattatttgaagaaaaccctattaacgcaagtagagtagatgctaaagcgattctttctgcacgattgagtaaatcaagacgattagaaaatctcattgctcagctccccggtgagaagagaaatggcttgtttgggaatctcattgctttgtcattgggattgacccctaattttaaatcaaattttgatttggcagaagatgctaaattacagctttcaaaagatacttacgatgatgatttagataatttattggcgcaaattggagatcaatatgctgatttgtttttggcagctaagaatttatcagatgctattttactttcagatatcctaagagtaaatagtgaaataactaaggctcccctatcagcttcaatgattaagcgctacgatgaacatcatcaagacttgactcttttaaaagctttagttcgacaacaacttccagaaaagtataaagaaatcttttttgatcaatcaaaaaacggatatgcaggttatattgatgggggagctagccaagaagaattttataaatttatcaaaccaattttagaaaaaatggatggtactgaggaattattggtgaaactaaatcgtgaagatttgctgcgcaagcaacggacctttgacaacggctctattccccatcaaattcacttgggtgagctgcatgctattttgagaagacaagaagacttttatccatttttaaaagacaatcgtgagaagattgaaaaaatcttgacttttcgaattccttattatgttggtccattggcgcgtggcaatagtcgttttgcatggatgactcggaagtctgaagaaacaattaccccatggaattttgaagaagttgtcgataaaggtgcttcagctcaatcatttattgaacgcatgacaaactttgataaaaatcttccaaatgaaaaagtactaccaaaacatagtttgctttatgagtattttacggtttataacgaattgacaaaggtcaaatatgttactgagggaatgcgaaaaccagcatttctttcaggtgaacagaagaaagccattgttgatttactcttcaaaacaaatcgaaaagtaaccgttaagcaattaaaagaagattatttcaaaaaaatagaatgttttgatagtgttgaaatttcaggagttgaagatagatttaatgcttcattaggcgcctaccatgatttgctaaaaattattaaagataaagattttttggataatgaagaaaatgaagatatcttagaggatattgttttaacattgaccttatttgaagatagggggatgattgaggaaagacttaaaacatatgctcacctctttgatgataaggtgatgaaacagcttaaacgtcgccgttatactggttggggacgtttgtctcgaaaattgattaatggtattagggataagcaatctggcaaaacaatattagattttttgaaatcagatggttttgccaatcgcaattttatgcagctgatccatgatgatagtttgacatttaaagaagatattcaaaaagcacaggtgtctggacaaggccatagtttacatgaacagattgctaacttagctggcagtcctgctattaaaaaaggtattttacagactgtaaaaattgttgatgaactggtcaaagtaatggggcataagccagaaaatatcgttattgaaatggcacgtgaaaatcagacaactcaaaagggccagaaaaattcgcgagagcgtatgaaacgaatcgaagaaggtatcaaagaattaggaagtcagattcttaaagagcatcctgttgaaaatactcaattgcaaaatgaaaagctctatctctattatctacaaaatggaagagacatgtatgtggaccaagaattagatattaatcgtttaagtgattatgatgtcgatcacattgttccacaaagtttcattaaagacgattcaatagacaataaggtactaacgcgttctgataaaaatcgtggtaaatcggataacgttccaagtgaagaagtagtcaaaaagatgaaaaactattggagacaacttctaaacgccaagttaatcactcaacgtaagtttgataatttaacgaaagctgaacgtggaggtttgagtgaacttgataaagctggttttatcaaacgccaattggttgaaactcgccaaatcactaagcatgtggcacaaattttggatagtcgcatgaatactaaatacgatgaaaatgataaacttattcgagaggttaaagtgattaccttaaaatctaaattagtttctgacttccgaaaagatttccaattctataaagtacgtgagattaacaattaccatcatgcccatgatgcgtatctaaatgccgtcgttggaactgctttgattaagaaatatccaaaacttgaatcggagtttgtctatggtgattataaagtttatgatgttcgtaaaatgattgctaagtctgagcaagaaataggcaaagcaaccgcaaaatatttcttttactctaatatcatgaacttcttcaaaacagaaattacacttgcaaatggagagattcgcaaacgccctctaatcgaaactaatggggaaactggagaaattgtctgggataaagggcgagattttgccacagtgcgcaaagtattgtccatgccccaagtcaatattgtcaagaaaacagaagtacagacaggcggattctccaaggagtcaattttaccaaaaagaaattcggacaagcttattgctcgtaaaaaagactgggatccaaaaaaatatggtggttttgatagtccaacggtagcttattcagtcctagtggttgctaaggtggaaaaagggaaatcgaagaagttaaaatccgttaaagagttactagggatcacaattatggaaagaagttcctttgaaaaaaatccgattgactttttagaagctaaaggatataaggaagttaaaaaagacttaatcattaaactacctaaatatagtctttttgagttagaaaacggtcgtaaacggatgctggctagtgccggagaattacaaaaaggaaatgagctggctctgccaagcaaatatgtgaattttttatatttagctagtcattatgaaaagttgaagggtagtccagaagataacgaacaaaaacaattgtttgtggagcagcataagcattatttagatgagattattgagcaaatcagtgaattttctaagcgtgttattttagcagatgccaatttagataaagttcttagtgcatataacaaacatagagacaaaccaatacgtgaacaagcagaaaatattattcatttatttacgttgacgaatcttggagctcccgctgcttttaaatattttgatacaacaattgatcgtaaacgatatacgtctacaaaagaagttttagatgccactcttatccatcaatccatcactggtctttatgaaacacgcattgatttgagtcagctaggaggtgactga

SEQ ID NO: 41 - protein, 1367 aa, Artificial Sequence
  Synthetic Polypeptide
MDKKYSIGLDIGTNSVGWAVITDDYKVPSKKFKVLGNTDRHSIKKNLIGALLFGSGETAEATRLKRTARRRYTRRKNRICYLQEIFSNEMAKVDDSFFHRLEESFLVEEDKKHERHPIFGNIVDEVAYHEKYPTIYHLRKKLADSTDKADLRLIYLALAHMIKFRGHFLIEGDLNPDNSDVDKLFIQLVQIYNQLFEENPINASRVDAKAILSARLSKSRRLENLIAQLPGEKRNGLFGNLIALSLGLTPNFKSNFDLAEDAKLQLSKDTYDDDLDNLLAQIGDQYADLFLAAKNLSDAILLSDILRVNSEITKAPLSASMIKRYDEHHQDLTLLKALVRQQLPEKYKEIFFDQSKNGYAGYIDGGASQEEFYKFIKPILEKMDGTEELLVKLNREDLLRKQRTFDNGSIPHQIHLGELHAILRRQEDFYPFLKDNREKIEKILTFRIPYYVGPLARGNSRFAWMTRKSEETITPWNFEEVVDKGASAQSFIERMTNFDKNLPNEKVLPKHSLLYEYFTVYNELTKVKYVTEGMRKPAFLSGEQKKAIVDLLFKTNRKVTVKQLKEDYFKKIECFDSVEISGVEDRFNASLGAYHDLLKIIKDKDFLDNEENEDILEDIVLTLTLFEDRGMIEERLKTYAHLFDDKVMKQLKRRRYTGWGRLSRKLINGIRDKQSGKTILDFLKSDGFANRNFMQLIHDDSLTFKEDIQKAQVSGQGHSLHEQIANLAGSPAIKKGILQTVKIVDELVKVMGHKPENIVIEMARENQTTQKGQKNSRERMKRIEEGIKELGSQILKEHPVENTQLQNEKLYLYYLQNGRDMYVDQELDINRLSDYDVDHIVPQSFIKDDSIDNKVLTRSDKNRGKSDNVPSEEVVKKMKNYWRQLLNAKLITQRKFDNLTKAERGGLSELDKAGFIKRQLVETRQITKHVAQILDSRMNTKYDENDKLIREVKVITLKSKLVSDFRKDFQFYKVREINNYHHAHDAYLNAVVGTALIKKYPKLESEFVYGDYKVYDVRKMIAKSEQEIGKATAKYFFYSNIMNFFKTEITLANGEIRKRPLIETNGETGEIVWDKGRDFATVRKVLSMPQVNIVKKTEVQTGGFSKESILPKRNSDKLIARKKDWDPKKYGGFDSPTVAYSVLVVAKVEKGKSKKLKSVKELLGITIMERSSFEKNPIDFLEAKGYKEVKKDLIIKLPKYSLFELENGRKRMLASAGELQKGNELALPSKYVNFLYLASHYEKLKGSPEDNEQKQLFVEQHKHYLDEIIEQISEFSKRVILADANLDKVLSAYNKHRDKPIREQAENIIHLFTLTNLGAPAAFKYFDTTIDRKRYTSTKEVLDATLIHQSITGLYETRIDLSQLGGD

SEQ ID NO: 42 - DNA, 100 bp, Artificial Sequence
  Synthetic Oligonucleotide
aacacatgggtcgacacaaacacaactcggcaggtacttgcagatgtagtctttccacatgggtcgacacaaacacaactcggcaggtatctcgtatgcc

SEQ ID NO: 43 - DNA, 10 bp, Artificial Sequence
  Synthetic Oligonucleotide
ctcggcaggt

SEQ ID NO: 44 - DNA, 43 bp, Artificial Sequence
  Synthetic Oligonucleotide
acttgcagatgtagtctttccacatgggtcgacacaaacacaa

SEQ ID NO: 45 - DNA, 12 bp, Artificial Sequence
  Synthetic Oligonucleotide
tgtgtttgtgtt

SEQ ID NO: 46 - DNA, 12 bp, Artificial Sequence
  Synthetic Oligonucleotide
agaagaagaaga

SEQ ID NO: 47 - DNA, 12 bp, Artificial Sequence
  Synthetic Oligonucleotide
ttctctttctct

SEQ ID NO: 48 - DNA, 12 bp, Artificial Sequence
  Synthetic Oligonucleotide
acacaaacacaa

SEQ ID NO: 49 - DNA, 43 bp, Artificial Sequence; identical to SEQ ID NO: 44
  Synthetic Oligonucleotide

SEQ ID NO: 50 - DNA, 31 bp, Artificial Sequence
  Synthetic Oligonucleotide
acttgcagatgtagtctttccacatgggtcg

SEQ ID NO: 51 - DNA, 100 bp, Artificial Sequence; identical to SEQ ID NO: 42
  Synthetic Oligonucleotide

SEQ ID NO: 52 - DNA, 162 bp, Artificial Sequence
  Synthetic Oligonucleotide
caatctcccgcatgcgctcagtcctcatctccctcaagcaggccccgctggtgcactgaagagccaccctgtgaaacactacatctgcaatatcttaatcctactcagtgaagctcttcacagtcattggattaattatgttgagttcttttggaccaaacc

SEQ ID NO: 53 - DNA, 20 bp, Artificial Sequence
  Synthetic Oligonucleotide
gctggtgcactgaagagcca

SEQ ID NO: 54 - DNA, 20 bp, Artificial Sequence
  Synthetic Oligonucleotide
aatatcttaatcctactcag

SEQ ID NO: 55 - DNA, 22 bp, Artificial Sequence
  Synthetic Oligonucleotide
ccctgtgaaacactacatctgc

SEQ ID NO: 56 - DNA, 22 bp, Artificial Sequence
  Synthetic Oligonucleotide
gcagatgtagtgtttcacaggg

SEQ ID NO: 57 - DNA, 23 bp, Artificial Sequence
  Synthetic Oligonucleotide
gcagatgtagtgtttccacaggg

SEQ ID NO: 58 - DNA, 23 bp, Artificial Sequence
  Synthetic Oligonucleotide
gcagatgtagtgtttccacaggg

SEQ ID NO: 59 - DNA, 23 bp, Artificial Sequence
  Synthetic Oligonucleotide
acatatgtagtatttccacaggg

SEQ ID NO: 60 - DNA, 23 bp, Artificial Sequence
  Synthetic Oligonucleotide
gcatatgtagtgtttccaaatgt

SEQ ID NO: 61 - DNA, 23 bp, Artificial Sequence
  Synthetic Oligonucleotide
ccagatgtagtattcccacaggg

SEQ ID NO: 62 - DNA, 23 bp, Artificial Sequence
  Synthetic Oligonucleotide
gcagttttagtgttttcacaggg

SEQ ID NO: 63 - DNA, 23 bp, Artificial Sequence
  Synthetic Oligonucleotide
gcagagttagtgtttccacacag

SEQ ID NO: 64 - DNA, 23 bp, Artificial Sequence
  Synthetic Oligonucleotide
gcagatggagggttttcacaggg

SEQ ID NO: 65 - DNA, 23 bp, Artificial Sequence
  Synthetic Oligonucleotide
ggaaatttagtgtttccacaggg

SEQ ID NO: 66 - DNA, 23 bp, Artificial Sequence
  Synthetic Oligonucleotide
aaagaagtagtatttccacatgg

SEQ ID NO: 67 - DNA, 23 bp, Artificial Sequence
  Synthetic Oligonucleotide
aaagatgtagtcattccacaagg

SEQ ID NO: 68 - DNA, 23 bp, Artificial Sequence
  Synthetic Oligonucleotide
aaatatgtagtctttccacaggg

SEQ ID NO: 69 - DNA, 23 bp, Artificial Sequence
  Synthetic Oligonucleotide
atagatgtagtgtttccaaagga

SEQ ID NO: 70 - DNA, 23 bp, Artificial Sequence
  Synthetic Oligonucleotide
ccagaggtagtgctcccacaggg

SEQ ID NO: 71 - DNA, 23 bp, Artificial Sequence
  Synthetic Oligonucleotide
ccagatgtgaggtttccacaagg

SEQ ID NO: 72 - DNA, 23 bp, Artificial Sequence
  Synthetic Oligonucleotide
ctacatgtagtgtttccatatgg

SEQ ID NO: 73 - DNA, 22 bp, Artificial Sequence
  Synthetic Oligonucleotide
tagatgaagtgcttccacatgg

SEQ ID NO: 74 - DNA, 23 bp, Artificial Sequence
  Synthetic Oligonucleotide
gaaaatggagtgtttacacatgg

SEQ ID NO: 75 - DNA, 23 bp, Artificial Sequence
  Synthetic Oligonucleotide
gcaaatgaagtgtcaccacaagg

SEQ ID NO: 76 - DNA, 23 bp, Artificial Sequence
  Synthetic Oligonucleotide
gcaaatgtattatttccactagg

SEQ ID NO: 77 - DNA, 23 bp, Artificial Sequence
  Synthetic Oligonucleotide
gcagatgtagcttttgtacatgg

SEQ ID NO: 78 - DNA, 23 bp, Artificial Sequence
  Synthetic Oligonucleotide
gcagcttaagtgttttcacatgg

SEQ ID NO: 79 - DNA, 23 bp, Artificial Sequence
  Synthetic Oligonucleotide
ttacatgtagtgtttacacacgg

SEQ ID NO: 80 - DNA, 23 bp, Artificial Sequence
  Synthetic Oligonucleotide
gaagaggaagtgtttgcccaggg

SEQ ID NO: 81 - DNA, 23 bp, Artificial Sequence
  Synthetic Oligonucleotide
gaagatgtggagttgacacatgg

SEQ ID NO: 82 - DNA, 23 bp, Artificial Sequence
  Synthetic Oligonucleotide
gcagaagtactgttgttacaagg

SEQ ID NO: 83 - DNA, 23 bp, Artificial Sequence
  Synthetic Oligonucleotide
gcagatgtggaattacaacaggg

SEQ ID NO: 84 - DNA, 23 bp, Artificial Sequence
  Synthetic Oligonucleotide
gcagtcatagtgtatacacatgg

SEQ ID NO: 85 - DNA, 23 bp, Artificial Sequence
  Synthetic Oligonucleotide
taagatgtagtatttccaaaagt

SEQ ID NO: 86 - DNA, 23 bp, Artificial Sequence
  Synthetic Oligonucleotide
gcagctggcatttctccacacgg

SEQ ID NO: 87 - DNA, 23 bp, Artificial Sequence
  Synthetic Oligonucleotide
ggagatctgatggttctacaagg

SEQ ID NO: 88 - DNA, 23 bp, Artificial Sequence
  Synthetic Oligonucleotide
taaaatgcagtgtatccatatgg

SEQ ID NO: 89 - DNA, 23 bp, Artificial Sequence
  Synthetic Oligonucleotide
gccagaatagtttttcaacaagg

SEQ ID NO: 90 - DNA, 23 bp, Artificial Sequence
  Synthetic Oligonucleotide
ttgtatttagagattgcacaagg

SEQ ID NO: 91 - DNA, 23 bp, Artificial Sequence
  Synthetic Oligonucleotide
agtcctcatctccctcaagcagg

SEQ ID NO: 92 - DNA, 23 bp, Artificial Sequence
  Synthetic Oligonucleotide
agtcctcaactccctcaagcagg

SEQ ID NO: 93 - DNA, 23 bp, Artificial Sequence
  Synthetic Oligonucleotide
agccctcatttccctcaagcagg

SEQ ID NO: 94 - DNA, 23 bp, Artificial Sequence
  Synthetic Oligonucleotide
actcctcatccccctcaagccgg

SEQ ID NO: 95 - DNA, 23 bp, Artificial Sequence
  Synthetic Oligonucleotide
agtcatcatctccctcaagcaga

SEQ ID NO: 96 - DNA, 23 bp, Artificial Sequence
  Synthetic Oligonucleotide
cgtcctcctctcccccaagcagg

SEQ ID NO: 97 - DNA, 23 bp, Artificial Sequence
  Synthetic Oligonucleotide
tgtcctcttctccctcaagcaga

SEQ ID NO: 98 - DNA, 23 bp, Artificial Sequence
  Synthetic Oligonucleotide
aagcttcatctctctcaagctgg

SEQ ID NO: 99 - DNA, 23 bp, Artificial Sequence
  Synthetic Oligonucleotide
agtactcttttccctcaggctgg

SEQ ID NO: 100 - DNA, 23 bp, Artificial Sequence
  Synthetic Oligonucleotide
agtcttaaattccctcaagcagg

SEQ ID NO: 101 - DNA, 23 bp, Artificial Sequence
  Synthetic Oligonucleotide
agtgctcatctaccagaagctgg

SEQ ID NO: 102 - DNA, 23 bp, Artificial Sequence
  Synthetic Oligonucleotide
cctcctcatctccctgcagcagg

SEQ ID NO: 103 - DNA, 23 bp, Artificial Sequence
  Synthetic Oligonucleotide
ctacatcatctccctcaagctgg

SEQ ID NO: 104 - DNA, 23 bp, Artificial Sequence
  Synthetic Oligonucleotide
ggtcctcatctccctaaaacaga

SEQ ID NO: 105 - DNA, 23 bp, Artificial Sequence
  Synthetic Oligonucleotide
tgtcctcatcggcctcaggcagg

SEQ ID NO: 106 - DNA, 23 bp, Artificial Sequence
  Synthetic Oligonucleotide
agacaccatctcccttgagctgg

SEQ ID NO: 107 - DNA, 23 bp, Artificial Sequence
  Synthetic Oligonucleotide
aggcatcatctacatcaagttgg

SEQ ID NO: 108 - DNA, 23 bp, Artificial Sequence
  Synthetic Oligonucleotide
agtaatcacttccatcaagccgg

SEQ ID NO: 109 - DNA, 23 bp, Artificial Sequence
  Synthetic Oligonucleotide
tcccctcacctccctaaagcagg

SEQ ID NO: 110 - DNA, 23 bp, Artificial Sequence
  Synthetic Oligonucleotide
tgtctttatttccctctagctgg

SEQ ID NO: 111 - DNA, 23 bp, Artificial Sequence
  Synthetic Oligonucleotide
agtcctcatctccctcaagcagg

SEQ ID NO: 112 - DNA, 23 bp, Artificial Sequence
  Synthetic Oligonucleotide
gcagatgtagtgtttccacaggg

SEQ ID NO: 113 - DNA, 23 bp, Artificial Sequence
  Synthetic Oligonucleotide
acatatgtagtatttccacaggg

SEQ ID NO: 114 - DNA, 23 bp, Artificial Sequence
  Synthetic Oligonucleotide
gcatatgtagtgtttccaaatgt

SEQ ID NO: 115 - DNA, 23 bp, Artificial Sequence
  Synthetic Oligonucleotide
ccagatgtagtattcccacaggg

SEQ ID NO: 116 - DNA, 23 bp, Artificial Sequence
  Synthetic Oligonucleotide
gcagttttagtgttttcacaggg

SEQ ID NO: 117 - DNA, 23 bp, Artificial Sequence
  Synthetic Oligonucleotide
gcagagttagtgtttccacacag

SEQ ID NO: 118 - DNA, 23 bp, Artificial Sequence
  Synthetic Oligonucleotide
gcagatggagggttttcacaggg

SEQ ID NO: 119 - DNA, 23 bp, Artificial Sequence
  Synthetic Oligonucleotide
ggaaatttagtgtttccacaggg

SEQ ID NO: 120 - DNA, 23 bp, Artificial Sequence
  Synthetic Oligonucleotide
aaagaagtagtatttccacatgg

SEQ ID NO: 121 - DNA, 23 bp, Artificial Sequence
  Synthetic Oligonucleotide
aaagatgtagtcattccacaagg

SEQ ID NO: 122 - DNA, 23 bp, Artificial Sequence
  Synthetic Oligonucleotide
aaatatgtagtctttccacaggg

SEQ ID NO: 123 - DNA, 23 bp, Artificial Sequence
  Synthetic Oligonucleotide
atagatgtagtgtttccaaagga

SEQ ID NO: 124 - DNA, 23 bp, Artificial Sequence
  Synthetic Oligonucleotide
ccagaggtagtgctcccacaggg

SEQ ID NO: 125 - DNA, 23 bp, Artificial Sequence
  Synthetic Oligonucleotide
ccagatgtgaggtttccacaagg

SEQ ID NO: 126 - DNA, 23 bp, Artificial Sequence
  Synthetic Oligonucleotide
ctacatgtagtgtttccatatgg

SEQ ID NO: 127 - DNA, 23 bp, Artificial Sequence
  Synthetic Oligonucleotide
ctagatgaagtgcttccacatgg

SEQ ID NO: 128 - DNA, 23 bp, Artificial Sequence
  Synthetic Oligonucleotide
gaaaatggagtgtttacacatgg

SEQ ID NO: 129 - DNA, 23 bp, Artificial Sequence
  Synthetic Oligonucleotide
gcaaatgaagtgtcaccacaagg

SEQ ID NO: 130 - DNA, 23 bp, Artificial Sequence
  Synthetic Oligonucleotide
gcaaatgtattatttccactagg

SEQ ID NO: 131 - DNA, 23 bp, Artificial Sequence
  Synthetic Oligonucleotide
gcagatgtagcttttgtacatgg

SEQ ID NO: 132 - DNA, 23 bp, Artificial Sequence
  Synthetic Oligonucleotide
gcagcttaagtgttttcacatgg

SEQ ID NO: 133 - DNA, 23 bp, Artificial Sequence
  Synthetic Oligonucleotide
ttacatgtagtgtttacacacgg

SEQ ID NO: 134 - DNA, 23 bp, Artificial Sequence
  Synthetic Oligonucleotide
gaagaggaagtgtttgcccaggg

SEQ ID NO: 135 - DNA, 23 bp, Artificial Sequence
  Synthetic Oligonucleotide
gaagatgtggagttgacacatgg

SEQ ID NO: 136 - DNA, 23 bp, Artificial Sequence
  Synthetic Oligonucleotide
gcagaagtactgttgttacaagg

SEQ ID NO: 137 - DNA, 23 bp, Artificial Sequence
  Synthetic Oligonucleotide
gcagatgtggaattacaacaggg

SEQ ID NO: 138 - DNA, 23 bp, Artificial Sequence
  Synthetic Oligonucleotide
gcagtcatagtgtatacacatgg

SEQ ID NO: 139 - DNA, 23 bp, Artificial Sequence
  Synthetic Oligonucleotide
taagatgtagtatttccaaaagt

SEQ ID NO: 140 - DNA, 23 bp, Artificial Sequence
  Synthetic Oligonucleotide
gcagctggcatttctccacacgg

SEQ ID NO: 141 - DNA, 23 bp, Artificial Sequence
  Synthetic Oligonucleotide
ggagatctgatggttctacaagg

SEQ ID NO: 142 - DNA, 23 bp, Artificial Sequence
  Synthetic Oligonucleotide
taaaatgcagtgtatccatatgg

SEQ ID NO: 143 - DNA, 23 bp, Artificial Sequence
  Synthetic Oligonucleotide
gccagaatagtttttcaacaagg

SEQ ID NO: 144 - DNA, 23 bp, Artificial Sequence
  Synthetic Oligonucleotide
ttgtatttagagattgcacaagg

SEQ ID NO: 145 - DNA, 23 bp, Artificial Sequence
  Synthetic Oligonucleotide
agtcctcatctccctcaagcagg

SEQ ID NO: 146 - DNA, 23 bp, Artificial Sequence
  Synthetic Oligonucleotide
agtcctcaactccctcaagcagg

SEQ ID NO: 147 - DNA, 23 bp, Artificial Sequence
  Synthetic Oligonucleotide
agccctcatttccctcaagcagg

SEQ ID NO: 148 - DNA, 23 bp, Artificial Sequence
  Synthetic Oligonucleotide
actcctcatccccctcaagccgg

SEQ ID NO: 149 - DNA, 23 bp, Artificial Sequence
  Synthetic Oligonucleotide
agtcatcatctccctcaagcaga

SEQ ID NO: 150 - DNA, 23 bp, Artificial Sequence
  Synthetic Oligonucleotide
cgtcctcctctcccccaagcagg

SEQ ID NO: 151 - DNA, 23 bp, Artificial Sequence
  Synthetic Oligonucleotide
tgtcctcttctccctcaagcaga

SEQ ID NO: 152 - DNA, 23 bp, Artificial Sequence
  Synthetic Oligonucleotide
aagcttcatctctctcaagctgg

SEQ ID NO: 153 - DNA, 23 bp, Artificial Sequence
  Synthetic Oligonucleotide
agtactcttttccctcaggctgg

SEQ ID NO: 154 - DNA, 23 bp, Artificial Sequence
  Synthetic Oligonucleotide
agtcttaaattccctcaagcagg

SEQ ID NO: 155 - DNA, 23 bp, Artificial Sequence
  Synthetic Oligonucleotide
agtgctcatctaccagaagctgg

SEQ ID NO: 156 - DNA, 23 bp, Artificial Sequence
  Synthetic Oligonucleotide
cctcctcatctccctgcagcagg

SEQ ID NO: 157 - DNA, 23 bp, Artificial Sequence
  Synthetic Oligonucleotide
ctacatcatctccctcaagctgg

SEQ ID NO: 158 - DNA, 23 bp, Artificial Sequence
  Synthetic Oligonucleotide
ggtcctcatctccctaaaacaga

SEQ ID NO: 159 - DNA, 23 bp, Artificial Sequence
  Synthetic Oligonucleotide
tgtcctcatcggcctcaggcagg

SEQ ID NO: 160 - DNA, 23 bp, Artificial Sequence
  Synthetic Oligonucleotide
agacaccatctcccttgagctgg

SEQ ID NO: 161 - DNA, 23 bp, Artificial Sequence
  Synthetic Oligonucleotide
aggcatcatctacatcaagttgg

SEQ ID NO: 162 - DNA, 23 bp, Artificial Sequence
  Synthetic Oligonucleotide
agtaatcacttccatcaagccgg

SEQ ID NO: 163 - DNA, 23 bp, Artificial Sequence
  Synthetic Oligonucleotide
tcccctcacctccctaaagcagg

SEQ ID NO: 164 - DNA, 23 bp, Artificial Sequence
  Synthetic Oligonucleotide
tgtctttatttccctctagctgg

SEQ ID NO: 165 - DNA, 23 bp, Artificial Sequence
  Synthetic Oligonucleotide
agtcctcatctccctcaagcagg

SEQ ID NO: 166 - DNA, 23 bp, Artificial Sequence
  Synthetic Oligonucleotide
agtcctcatctccctcaagcagg

SEQ ID NO: 167 - DNA, 24 bp, Artificial Sequence
  Synthetic Oligonucleotide
agtcctcatctccctcaaagcagg

SEQ ID NO: 168 - DNA, 22 bp, Artificial Sequence
  Synthetic Oligonucleotide
agtcctcatctccctcagcagg

SEQ ID NO: 169 - DNA, 24 bp, Artificial Sequence
  Synthetic Oligonucleotide
agtcctcatctccctcatagcagg

SEQ ID NO: 170 - DNA, 15 bp, Artificial Sequence
  Synthetic Oligonucleotide
agtcctcatagcagg

SEQ ID NO: 171 - DNA, 17 bp, Artificial Sequence
  Synthetic Oligonucleotide
agtcctcatctagcagg

SEQ ID NO: 172 - DNA, 14 bp, Artificial Sequence
  Synthetic Oligonucleotide
agtcctcaagcagg

SEQ ID NO: 173 - DNA, 51 bp, Artificial Sequence
  Synthetic Oligonucleotide
agtcctcatctccctcaaaggcagtgtttgttacttgagtttgtcagcagg

SEQ ID NO: 174 - DNA, 25 bp, Artificial Sequence
  Synthetic Oligonucleotide
agtcctcatctccctcattagcagg

SEQ ID NO: 175 - DNA, 65 bp, Artificial Sequence
  Synthetic Oligonucleotide
agtcctcatctccctcagggcttgtttacagctcacctttgaatttgcacaagcgtgcaagcagg

SEQ ID NO: 176 - DNA, 21 bp, Artificial Sequence
  Synthetic Oligonucleotide
agtcctcatctccctagcagg

SEQ ID NO: 177 - DNA, 21 bp, Artificial Sequence
  Synthetic Oligonucleotide
agtcctcatccctcaagcagg

SEQ ID NO: 178 - DNA, 22 bp, Artificial Sequence
  Synthetic Oligonucleotide
agtcctcatctccctaagcagg

SEQ ID NO: 179 - DNA, 23 bp, Artificial Sequence
  Synthetic Oligonucleotide
agtcctcaactccctcaagcagg

SEQ ID NO: 180 - DNA, 24 bp, Artificial Sequence
  Synthetic Oligonucleotide
agtcctcaactccctcaaagcagg

SEQ ID NO: 181 - DNA, 17 bp, Artificial Sequence
  Synthetic Oligonucleotide
agtcctcaactccctca

SEQ ID NO: 182 - DNA, 22 bp, Artificial Sequence
  Synthetic Oligonucleotide
agtcctcaactccctcagcagg

SEQ ID NO: 183 - DNA, 56 bp, Artificial Sequence
  Synthetic Oligonucleotide
agtcctcaactccctcaagaaaggtgttgaaaatcagaaagagagaaacaagcagg

SEQ ID NO: 184 - DNA, 62 bp, Artificial Sequence
  Synthetic Oligonucleotide
agtcctcaactccctcaatctacggtccattcccgtttccactcaccttgcgccgcagcagg

SEQ ID NO: 185 - DNA, 22 bp, Artificial Sequence
  Synthetic Oligonucleotide
agtcctcaactccctaagcagg

SEQ ID NO: 186 - DNA, 66 bp, Artificial Sequence
  Synthetic Oligonucleotide
agtcctcaactccctcaaccaactttaacatcctgctggttctgtcattaataagttgaaagcagg

SEQ ID NO: 187 - DNA, 64 bp, Artificial Sequence
  Synthetic Oligonucleotide
agtcctcaactccctcacagcaaataaaaaagttgtttatgcatattcagataagcaaagcagg

SEQ ID NO: 188 - DNA, 21 bp, Artificial Sequence
  Synthetic Oligonucleotide
agtcctcaactcccaagcagg

SEQ ID NO: 189 - DNA, 23 bp, Artificial Sequence
  Synthetic Oligonucleotide
actcctcatccccctcaagccgg

SEQ ID NO: 190 - DNA, 24 bp, Artificial Sequence
  Synthetic Oligonucleotide
actcctcatccccctcaaagccgg

SEQ ID NO: 191 - DNA, 24 bp, Artificial Sequence
  Synthetic Oligonucleotide
actcctcatccccctcagagccgg

SEQ ID NO: 192 - DNA, 13 bp, Artificial Sequence
  Synthetic Oligonucleotide
actcctcagccgg

SEQ ID NO: 193 - DNA, 25 bp, Artificial Sequence
  Synthetic Oligonucleotide
actcctcatccccctcaaaagccgg

SEQ ID NO: 194 - DNA, 25 bp, Artificial Sequence
  Synthetic Oligonucleotide
actcctcatccccctcagcagccgg

SEQ ID NO: 195 - DNA, 24 bp, Artificial Sequence
  Synthetic Oligonucleotide
actcctcatccccctcatagccgg

SEQ ID NO: 196 - DNA, 24 bp, Artificial Sequence
  Synthetic Oligonucleotide
actcctcatccccctcatccccgg

SEQ ID NO: 197 - DNA, 18 bp, Artificial Sequence
  Synthetic Oligonucleotide
actcctcatcccagccgg

SEQ ID NO: 198 - DNA, 22 bp, Artificial Sequence
  Synthetic Oligonucleotide
actcctcatccccctaagccgg

SEQ ID NO: 199 - DNA, 25 bp, Artificial Sequence
  Synthetic Oligonucleotide
actcctcatccccctcaatagccgg

SEQ ID NO: 200 - DNA, 25 bp, Artificial Sequence
  Synthetic Oligonucleotide
actcctcacccccctcagcagccgg

SEQ ID NO: 201 - DNA, 23 bp, Artificial Sequence
  Synthetic Oligonucleotide
gcagatgtagtgtttccacaggg

SEQ ID NO: 202 - DNA, 22 bp, Artificial Sequence
  Synthetic Oligonucleotide
gcagatgtagtgtttcacaggg

SEQ ID NO: 203 - DNA, 24 bp, Artificial Sequence
  Synthetic Oligonucleotide
gcagatgtagtgtttcccacaggg

SEQ ID NO: 204 - DNA, 19 bp, Artificial Sequence
  Synthetic Oligonucleotide
gcagatgtagtgcacaggg

SEQ ID NO: 205 - DNA, 22 bp, Artificial Sequence
  Synthetic Oligonucleotide
gcagatgtagtgtttcccaggg

SEQ ID NO: 206 - DNA, 16 bp, Artificial Sequence
  Synthetic Oligonucleotide
gcagatgtacacaggg

SEQ ID NO: 207 - DNA, 20 bp, Artificial Sequence
  Synthetic Oligonucleotide
gcagatgtagtgtcacaggg

SEQ ID NO: 208 - DNA, 21 bp, Artificial Sequence
  Synthetic Oligonucleotide
gcagatgtagtgttcacaggg

SEQ ID NO: 209 - DNA, 21 bp, Artificial Sequence
  Synthetic Oligonucleotide
gcagatgtagtgtttccaggg

SEQ ID NO: 210 - DNA, 18 bp, Artificial Sequence
  Synthetic Oligonucleotide
gcagatgtagtcacaggg

SEQ ID NO: 211 - DNA, 12 bp, Artificial Sequence
  Synthetic Oligonucleotide
gcagatgtaggg

SEQ ID NO: 212 - DNA, 23 bp, Artificial Sequence
  Synthetic Oligonucleotide
acatatgtagtatttccacaggg

SEQ ID NO: 213 - DNA, 24 bp, Artificial Sequence
  Synthetic Oligonucleotide
acatatgtagtatttcccacaggg

SEQ ID NO: 214 - DNA, 22 bp, Artificial Sequence
  Synthetic Oligonucleotide
acatatgtagtatttcacaggg

SEQ ID NO: 215 - DNA, 21 bp, Artificial Sequence
  Synthetic Oligonucleotide
acatatgtagtatttccaggg

SEQ ID NO: 216 - DNA, 13 bp, Artificial Sequence
  Synthetic Oligonucleotide
acatatcacaggg

SEQ ID NO: 217 - DNA, 11 bp, Artificial Sequence
  Synthetic Oligonucleotide
acatcacaggg

SEQ ID NO: 218 - DNA, 18 bp, Artificial Sequence
  Synthetic Oligonucleotide
acatatgtagtcacaggg

SEQ ID NO: 219 - DNA, 17 bp, Artificial Sequence
  Synthetic Oligonucleotide
acatatgtagtatttcc

SEQ ID NO: 220 - DNA, 12 bp, Artificial Sequence
  Synthetic Oligonucleotide
acatatgtaggg

SEQ ID NO: 221 - DNA, 17 bp, Artificial Sequence
  Synthetic Oligonucleotide
acatatgtagcacaggg

SEQ ID NO: 222 - DNA, 23 bp, Artificial Sequence
  Synthetic Oligonucleotide
ccagatgtagtattcccacaggg

SEQ ID NO: 223 - DNA, 24 bp, Artificial Sequence
  Synthetic Oligonucleotide
ccagatgtagtattccccacaggg

SEQ ID NO: 224 - DNA, 19 bp, Artificial Sequence
  Synthetic Oligonucleotide
ccagatgtagtatacaggg

SEQ ID NO: 225 - DNA, 20 bp, Artificial Sequence
  Synthetic Oligonucleotide
ccagatgtagtatcacaggg

SEQ ID NO: 226 - DNA, 26 bp, Artificial Sequence
  Synthetic Oligonucleotide
ccagatgtagtattcccaacacaggg

SEQ ID NO: 227 - DNA, 21 bp, Artificial Sequence
  Synthetic Oligonucleotide
ccagatgtagtattcacaggg

SEQ ID NO: 228 - DNA, 21 bp, Artificial Sequence
  Synthetic Oligonucleotide
ccagatgtagtattcccaggg

SEQ ID NO: 229 - DNA, 22 bp, Artificial Sequence
  Synthetic Oligonucleotide
ccagatgtagtattccacaggg

SEQ ID NO: 230 - DNA, 23 bp, Artificial Sequence
  Synthetic Oligonucleotide
ctagatgaagtgcttccacatgg

SEQ ID NO: 231 - DNA, 24 bp, Artificial Sequence
  Synthetic Oligonucleotide
ctagatgaagtgcttcccacatgg

SEQ ID NO: 232 - DNA, 22 bp, Artificial Sequence
  Synthetic Oligonucleotide
ctagatgaagtgcttcacatgg

SEQ ID NO: 233 - DNA, 12 bp, Artificial Sequence
  Synthetic Oligonucleotide
ctagatgaagtg

SEQ ID NO: 234 - DNA, 25 bp, Artificial Sequence
  Synthetic Oligonucleotide
ctagatgaagtgcttccacacatgg

SEQ ID NO: 235 - DNA, 21 bp, Artificial Sequence
  Synthetic Oligonucleotide
ctagatgaagtgcttccatgg

SEQ ID NO: 236 - DNA, 22 bp, Artificial Sequence
  Synthetic Oligonucleotide
ctagatgaagtgcttcccatgg

SEQ ID NO: 237 - DNA, 56 bp, Artificial Sequence
  Synthetic Oligonucleotide
taatacgactcactataggagtcctcatctccctcaagcgttttagagctatgctg

SEQ ID NO: 238 - DNA, 56 bp, Artificial Sequence
  Synthetic Oligonucleotide
taatacgactcactataggctccctcaagcaggccccgcgttttagagctatgctg

SEQ ID NO: 239 - DNA, 56 bp, Artificial Sequence
  Synthetic Oligonucleotide
taatacgactcactataggtgtgaagagcttcactgagtgttttagagctatgctg

SEQ ID NO: 240 - DNA, 56 bp, Artificial Sequence
  Synthetic Oligonucleotide
taatacgactcactatagggcagatgtagtgtttccacagttttagagctatgctg

SEQ ID NO: 241 - DNA, 55 bp, Artificial Sequence
  Synthetic Oligonucleotide
gataacggactagccttattttaacttgctatgcttttcagcatagctctaaaac

SEQ ID NO: 242 - DNA, 81 bp, Artificial Sequence
  Synthetic Oligonucleotide
cggactagccttattttaacttgctatttctagctctaaaacgcttgagggagatgaggactcctatagtgagtcgtatta

SEQ ID NO: 243 - DNA, 81 bp, Artificial Sequence
  Synthetic Oligonucleotide
cggactagccttattttaacttgctatttctagctctaaaacgcggggcctgcttgagggagcctatagtgagtcgtatta

SEQ ID NO: 244 - DNA, 81 bp, Artificial Sequence
  Synthetic Oligonucleotide
cggactagccttattttaacttgctatttctagctctaaaacactcagtgaagctcttcacacctatagtgagtcgtatta

SEQ ID NO: 245 - DNA, 81 bp, Artificial Sequence
  Synthetic Oligonucleotide
cggactagccttattttaacttgctatttctagctctaaaactgtggaaacactacatctgccctatagtgagtcgtatta

SEQ ID NO: 246 - DNA, 19 bp, Artificial Sequence
  Synthetic Oligonucleotide
taatacgactcactatagg

SEQ ID NO: 247 - DNA, 53 bp, Artificial Sequence
  Synthetic Oligonucleotide
  misc_feature (7)..(10): n is a, c, g, or t
  misc_feature (13)..(13): n is a, c, g, or t
  misc_feature (34)..(37): n is a, c, g, or t
aacacannnnccngcttgagggagatgaggactnnnnacctgccgagaacaca

SEQ ID NO: 248 - DNA, 53 bp, Artificial Sequence
  Synthetic Oligonucleotide
  misc_feature (7)..(10): n is a, c, g, or t
  misc_feature (13)..(13): n is a, c, g, or t
  misc_feature (34)..(37): n is a, c, g, or t
tcttctnnnnccngcggggcctgcttgagggagnnnnacctgccgagtcttct

SEQ ID NO: 249 - DNA, 53 bp, Artificial Sequence
  Synthetic Oligonucleotide
  misc_feature (7)..(10): n is a, c, g, or t
  misc_feature (13)..(13): n is a, c, g, or t
  misc_feature (34)..(37): n is a, c, g, or t
agagaannnnccnactcagtgaagctcttcacannnnacctgccgagagagaa

SEQ ID NO: 250 - DNA, 53 bp, Artificial Sequence
  Synthetic Oligonucleotide
  misc_feature (7)..(10): n is a, c, g, or t
  misc_feature (13)..(13): n is a, c, g, or t
  misc_feature (34)..(37): n is a, c, g, or t
ttgtgtnnnnccntgtggaaacactacatctgcnnnnacctgccgagttgtgt

SEQ ID NO: 251 - DNA, 29 bp, Artificial Sequence
  Synthetic Oligonucleotide
ctagcagtcctcatctccctcaagcaggc

SEQ ID NO: 252 - DNA, 29 bp, Artificial Sequence
  Synthetic Oligonucleotide
agctgcctgcttgagggagatgaggactg

SEQ ID NO: 253 - DNA, 29 bp, Artificial Sequence
  Synthetic Oligonucleotide
ctagtctccctcaagcaggccccgctggt

SEQ ID NO: 254 - DNA, 29 bp, Artificial Sequence
  Synthetic Oligonucleotide
agctaccagcggggcctgcttgagggaga

SEQ ID NO: 255 - DNA, 29 bp, Artificial Sequence
  Synthetic Oligonucleotide
ctagctgtgaagagcttcactgagtagga

SEQ ID NO: 256 - DNA, 29 bp, Artificial Sequence
  Synthetic Oligonucleotide
agcttcctactcagtgaagctcttcacag

SEQ ID NO: 257 - DNA, 29 bp, Artificial Sequence
  Synthetic Oligonucleotide
ctagtgcagatgtagtgtttccacagggt

SEQ ID NO: 258 - DNA, 29 bp, Artificial Sequence
  Synthetic Oligonucleotide
agctaccctgtggaaacactacatctgca

SEQ ID NO: 259 - DNA, 26 bp, Artificial Sequence
  Synthetic Oligonucleotide
gcgacacggaaatgttgaatactcat

SEQ ID NO: 260 - DNA, 25 bp, Artificial Sequence
  Synthetic Oligonucleotide
ggagtcaggcaactatggatgaacg

SEQ ID NO: 261 - DNA, 60 bp, Artificial Sequence
  Synthetic Oligonucleotide
actgtgaagagcttcactgagtaggattaagatattgcagatgtagtgtttccacagggt

SEQ ID NO: 262 - DNA, 60 bp, Artificial Sequence
  Synthetic Oligonucleotide
actgtgaagagcttcactgagtaggattaagatattgaagatgtagtgtttccacagggt

SEQ ID NO: 263 - DNA, 60 bp, Artificial Sequence
  Synthetic Oligonucleotide
actgtgaagagcttcactgagtaggattaagatattgaagatgtagtgtttccactgggt

SEQ ID NO: 264 - DNA, 60 bp, Artificial Sequence
  Synthetic Oligonucleotide
actgtgaagagcttcactgagtaggattaagatattgcagatggagggtttccacagggt

SEQ ID NO: 265 - DNA, 60 bp, Artificial Sequence
  Synthetic Oligonucleotide
actgtgaagagcttcactgagtaggattaagatattgcagatgtagtgttaccagagggt

SEQ ID NO: 266 - DNA, 60 bp, Artificial Sequence
  Synthetic Oligonucleotide
actgtgaagagcttcactgagtaggattaagatattggggatgtagtgtttccactgggt

SEQ ID NO: 267 - DNA, 60 bp, Artificial Sequence
  Synthetic Oligonucleotide
tccctcaagcaggccccgctggtgcactgaagagccaccctgtggaaacactacatctgc

SEQ ID NO: 268 - DNA, 60 bp, Artificial Sequence
  Synthetic Oligonucleotide
tccctcaagcaggccccgctggtgcactgaagagccaccctgtggaaacactacatcttc

SEQ ID NO: 269 - DNA, 60 bp, Artificial Sequence
  Synthetic Oligonucleotide
tccctcaagcaggccccgctggtgcactgaagagccacccagtggaaacactacatcttc

SEQ ID NO: 270 - DNA, 60 bp, Artificial Sequence
  Synthetic Oligonucleotide
tccctcaagcaggccccgctggtgcactgaagagccaccctgtggaaaccctccatctgc

SEQ ID NO: 271 - DNA, 60 bp, Artificial Sequence
  Synthetic Oligonucleotide
tccctcaagcaggccccgctggtgcactgaagagccaccctctggtaacactacatctgc

SEQ ID NO: 272 - DNA, 60 bp, Artificial Sequence
  Synthetic Oligonucleotide
tccctcaagcaggccccgctggtgcactgaagagccacccagtggaaacactacatcccc

SEQ ID NO: 273 - DNA, 62 bp, Artificial Sequence
  Synthetic Oligonucleotide
aatgatacggcgaccaccgagatctacactctttccctacacgacgctcttccgatctaaca

SEQ ID NO: 274 - DNA, 49 bp, Artificial Sequence
  Synthetic Oligonucleotide
tgttagatcggaagagcgtcgtgtagggaaagagtgtagatctcggtgg

SEQ ID NO: 275 - DNA, 62 bp, Artificial Sequence
  Synthetic Oligonucleotide
aatgatacggcgaccaccgagatctacactctttccctacacgacgctcttccgatctttca

SEQ ID NO: 276 - DNA, 49 bp, Artificial Sequence
  Synthetic Oligonucleotide
tgaaagatcggaagagcgtcgtgtagggaaagagtgtagatctcggtgg

SEQ ID NO: 277 - DNA, 58 bp, Artificial Sequence
  Synthetic Oligonucleotide
aatgatacggcgaccaccgagatctacactctttccctacacgacgctcttccgatct

SEQ ID NO: 278 - DNA, 45 bp, Artificial Sequence
  Synthetic Oligonucleotide
agatcggaagagcgtcgtgtagggaaagagtgtagatctcggtgg

SEQ ID NO: 279 - DNA, 15 bp, Artificial Sequence
  Synthetic Oligonucleotide
gacggcatacgagat

SEQ ID NO: 280 - DNA, 28 bp, Artificial Sequence
  Synthetic Oligonucleotide
aacaatctcgtatgccgtcttctgcttg

SEQ ID NO: 281 - DNA, 28 bp, Artificial Sequence
  Synthetic Oligonucleotide
tcttatctcgtatgccgtcttctgcttg

SEQ ID NO: 282 - DNA, 28 bp, Artificial Sequence
  Synthetic Oligonucleotide
agagatctcgtatgccgtcttctgcttg

SEQ ID NO: 283 - DNA, 28 bp, Artificial Sequence
  Synthetic Oligonucleotide
ttgtatctcgtatgccgtcttctgcttg

SEQ ID NO: 284 - DNA, 40 bp, Artificial Sequence
  Synthetic Oligonucleotide
caagcagaagacggcatacgagattgtgttctcggcaggt

SEQ ID NO: 285 - DNA, 40 bp, Artificial Sequence
  Synthetic Oligonucleotide
caagcagaagacggcatacgagatagaagactcggcaggt

SEQ ID NO: 286 - DNA, 40 bp, Artificial Sequence
  Synthetic Oligonucleotide
caagcagaagacggcatacgagatttctctctcggcaggt

SEQ ID NO: 287 - DNA, 40 bp, Artificial Sequence
  Synthetic Oligonucleotide
caagcagaagacggcatacgagatacacaactcggcaggt

SEQ ID NO: 288 - DNA, 20 bp, Artificial Sequence
  Synthetic Oligonucleotide
aatgatacggcgaccaccga

SEQ ID NO: 289 - DNA, 82 bp, Artificial Sequence
  Synthetic Oligonucleotide
  misc_feature (59)..(62): n is a, c, g, or t
aatgatacggcgaccaccgagatctacactctttccctacacgacgctcttccgatctnnnnacctacctgccgagaacaca

SEQ ID NO: 290 - DNA, 82 bp, Artificial Sequence
  Synthetic Oligonucleotide
  misc_feature (59)..(62): n is a, c, g, or t
aatgatacggcgaccaccgagatctacactctttccctacacgacgctcttccgatctnnnnacctacctgccgagtcttct

SEQ ID NO: 291 - DNA, 82 bp, Artificial Sequence
  Synthetic Oligonucleotide
  misc_feature (59)..(62): n is a, c, g, or t
aatgatacggcgaccaccgagatctacactctttccctacacgacgctcttccgatctnnnnacctacctgccgagagagaa

SEQ ID NO: 292 - DNA, 82 bp, Artificial Sequence
  Synthetic Oligonucleotide
  misc_feature (59)..(62): n is a, c, g, or t
aatgatacggcgaccaccgagatctacactctttccctacacgacgctcttccgatctnnnnacctacctgccgagttgtgt

SEQ ID NO: 293 - DNA, 24 bp, Artificial Sequence
  Synthetic Oligonucleotide
caagcagaagacggcatacgagat

SEQ ID NO: 294 - DNA, 53 bp, Artificial Sequence
  Synthetic Oligonucleotide
acactctttccctacacgacgctcttccgatctcaagtctagcaagcaggcca

SEQ ID NO: 295 - DNA, 53 bp, Artificial Sequence
  Synthetic Oligonucleotide
acactctttccctacacgacgctcttccgatctcaggcactgagtgggaaagt

SEQ ID NO: 296 - DNA, 53 bp, Artificial Sequence
  Synthetic Oligonucleotide
acactctttccctacacgacgctcttccgatcttaaccccaagtcagcaagca

SEQ ID NO: 297 - DNA, 53 bp, Artificial Sequence
  Synthetic Oligonucleotide
acactctttccctacacgacgctcttccgatctttgctggtcaataccctggc

SEQ ID NO: 298 - DNA, 53 bp, Artificial Sequence
  Synthetic Oligonucleotide
acactctttccctacacgacgctcttccgatcttgagtacccctgaaatgggc

SEQ ID NO: 299 - DNA, 53 bp, Artificial Sequence
  Synthetic Oligonucleotide
acactctttccctacacgacgctcttccgatcttcgctaccaatcagggcttt

SEQ ID NO: 300 - DNA, 53 bp, Artificial Sequence
  Synthetic Oligonucleotide
acactctttccctacacgacgctcttccgatctccattgccacttgtttgcat

SEQ ID NO: 301 - DNA, 53 bp, Artificial Sequence
  Synthetic Oligonucleotide
acactctttccctacacgacgctcttccgatctcctacccccacaactttgct

SEQ ID NO: 302 - DNA, 53 bp, Artificial Sequence
  Synthetic Oligonucleotide
acactctttccctacacgacgctcttccgatctgtgtacatccagtgcaccca

SEQ ID NO: 303 - DNA, 57 bp, Artificial Sequence
  Synthetic Oligonucleotide
acactctttccctacacgacgctcttccgatcttcggaaaggactttgaatacttgt

SEQ ID NO: 304 - DNA, 53 bp, Artificial Sequence
  Synthetic Oligonucleotide
acactctttccctacacgacgctcttccgatctcggcccaagacctcattcac

SEQ ID NO: 305 - DNA, 53 bp, Artificial Sequence
  Synthetic Oligonucleotide
acactctttccctacacgacgctcttccgatctgtcctctctggggcagaagt

SEQ ID NO: 306 - DNA, 55 bp, Artificial Sequence
  Synthetic Oligonucleotide
acactctttccctacacgacgctcttccgatctagctgagtcatgagttgtctcc

SEQ ID NO: 307 - DNA, 53 bp, Artificial Sequence
  Synthetic Oligonucleotide
acactctttccctacacgacgctcttccgatctctgccagcttctcacaccat

SEQ ID NO: 308 - DNA, 53 bp, Artificial Sequence
  Synthetic Oligonucleotide
acactctttccctacacgacgctcttccgatctctgaaggacaaaggcgggaa

SEQ ID NO: 309 - DNA, 53 bp, Artificial Sequence
  Synthetic Oligonucleotide
acactctttccctacacgacgctcttccgatctaaggtgctaaaggctccacg

SEQ ID NO: 310 - DNA, 53 bp, Artificial Sequence
  Synthetic Oligonucleotide
acactctttccctacacgacgctcttccgatctgaccattggtgagcccagag

SEQ ID NO: 311 - DNA, 53 bp, Artificial Sequence
  Synthetic Oligonucleotide
acactctttccctacacgacgctcttccgatcttttttcgggcaactgctcac

SEQ ID NO: 312 - DNA, 53 bp, Artificial Sequence
  Synthetic Oligonucleotide
acactctttccctacacgacgctcttccgatctgcaagccttctctcctcaga

SEQ ID NO: 313 - DNA, 54 bp, Artificial Sequence
  Synthetic Oligonucleotide
acactctttccctacacgacgctcttccgatctacacaaacttccctgagaccc

SEQ ID NO: 314 - DNA, 53 bp, Artificial Sequence
  Synthetic Oligonucleotide
acactctttccctacacgacgctcttccgatcttgagttagccctgctgttca

SEQ ID NO: 315 - DNA, 55 bp, Artificial Sequence
  Synthetic Oligonucleotide
acactctttccctacacgacgctcttccgatcttgaagagcttcactgagtagga

SEQ ID NO: 316 - DNA, 54 bp, Artificial Sequence
  Synthetic Oligonucleotide
acactctttccctacacgacgctcttccgatcttccccttacagccaatttcgt

SEQ ID NO: 317 - DNA, 58 bp, Artificial Sequence
  Synthetic Oligonucleotide
acactctttccctacacgacgctcttccgatcttgctgatgaaatgcaattaagaggt

SEQ ID NO: 318 - DNA, 53 bp, Artificial Sequence
  Synthetic Oligonucleotide
acactctttccctacacgacgctcttccgatctggtccctgcaagccagtatg

SEQ ID NO: 319 - DNA, 55 bp, Artificial Sequence
  Synthetic Oligonucleotide
acactctttccctacacgacgctcttccgatctatcaaagccttgtatcacagtt

SEQ ID NO: 320 - DNA, 54 bp, Artificial Sequence
  Synthetic Oligonucleotide
acactctttccctacacgacgctcttccgatctcccaaataatgcaggagccaa

SEQ ID NO: 321 - DNA, 55 bp, Artificial Sequence
  Synthetic Oligonucleotide
acactctttccctacacgacgctcttccgatctctgcctttagtgggacagactt

SEQ ID NO: 322 - DNA, 54 bp, Artificial Sequence
  Synthetic Oligonucleotide
acactctttccctacacgacgctcttccgatctagtaaccctagtagccctcca

SEQ ID NO: 323 - DNA, 54 bp, Artificial Sequence
  Synthetic Oligonucleotide
acactctttccctacacgacgctcttccgatctcattgcagtgagccgagattg

SEQ ID NO: 324 - DNA, 54 bp, Artificial Sequence
  Synthetic Oligonucleotide
acactctttccctacacgacgctcttccgatcttggcaaagttcacttccatgt

SEQ ID NO: 325 - DNA, 53 bp, Artificial Sequence
  Synthetic Oligonucleotide
acactctttccctacacgacgctcttccgatcttgctctgtgatgtctgccac

SEQ ID NO: 326 - DNA, 55 bp, Artificial Sequence
  Synthetic Oligonucleotide
acactctttccctacacgacgctcttccgatcttgtgtaggattgtgaaccagca

SEQ ID NO: 327 - DNA, 53 bp, Artificial Sequence
  Synthetic Oligonucleotide
acactctttccctacacgacgctcttccgatcttcccagcccagcatttttct

SEQ ID NO: 328 - DNA, 53 bp, Artificial Sequence
  Synthetic Oligonucleotide
acactctttccctacacgacgctcttccgatctaggttgctttgtgcacagtc

SEQ ID NO: 329 - DNA, 53 bp, Artificial Sequence
  Synthetic Oligonucleotide
acactctttccctacacgacgctcttccgatctcctggcttgggatgttggaa

SEQ ID NO: 330 - DNA, 53 bp, Artificial Sequence
  Synthetic Oligonucleotide
acactctttccctacacgacgctcttccgatctttgcccaaggtcatactgct

SEQ ID NO: 331 - DNA, 56 bp, Artificial Sequence
  Synthetic Oligonucleotide
acactctttccctacacgacgctcttccgatctacccactaggtagccataatcca

SEQ ID NO: 332 - DNA, 53 bp, Artificial Sequence
  Synthetic Oligonucleotide
acactctttccctacacgacgctcttccgatctcggtcatgtcgcttggaaga

SEQ ID NO: 333 - DNA, 56 bp, Artificial Sequence
  Synthetic Oligonucleotide
acactctttccctacacgacgctcttccgatctttggcccatattgctttatgctg

SEQ ID NO: 334 - DNA, 53 bp, Artificial Sequence
  Synthetic Oligonucleotide
acactctttccctacacgacgctcttccgatctattaggggttggctgcatga

SEQ ID NO: 335 - DNA, 53 bp, Artificial Sequence
  Synthetic Oligonucleotide
acactctttccctacacgacgctcttccgatctccaagacgtgttgcatgctg

SEQ ID NO: 336 - DNA, 57 bp, Artificial Sequence
  Synthetic Oligonucleotide
acactctttccctacacgacgctcttccgatcttgggaggtgataaattccctaaat

SEQ ID NO: 337 - DNA, 53 bp, Artificial Sequence
  Synthetic Oligonucleotide
acactctttccctacacgacgctcttccgatctccagagacaaaggtggggag

SEQ ID NO: 338 - DNA, 56 bp, Artificial Sequence
  Synthetic Oligonucleotide
acactctttccctacacgacgctcttccgatcttcatacagaagagcaaagtacca

SEQ ID NO: 339 - DNA, 53 bp, Artificial Sequence
  Synthetic Oligonucleotide
acactctttccctacacgacgctcttccgatctcaaagaggggtatcgggagc

SEQ ID NO: 340 - DNA, 57 bp, Artificial Sequence
  Synthetic Oligonucleotide
acactctttccctacacgacgctcttccgatctaaatggaagaaccaagtagatgaa

SEQ ID NO: 341 - DNA, 55 bp, Artificial Sequence
  Synthetic Oligonucleotide
acactctttccctacacgacgctcttccgatctttttggttgacagatggccaca

SEQ ID NO: 342 - DNA, 58 bp, Artificial Sequence
  Synthetic Oligonucleotide
acactctttccctacacgacgctcttccgatcttcttacttgtgtgattttagaacaa

SEQ ID NO: 343 - DNA, 53 bp, Artificial Sequence
  Synthetic Oligonucleotide
acactctttccctacacgacgctcttccgatctgatggttcatgcagagggct

SEQ ID NO: 344 - DNA, 53 bp, Artificial Sequence
  Synthetic Oligonucleotide
acactctttccctacacgacgctcttccgatctgctggtctttcctgagctgt

SEQ ID NO: 345 - DNA, 55 bp, Artificial Sequence
  Synthetic Oligonucleotide
acactctttccctacacgacgctcttccgatctctccatcagatacctgtaccca

SEQ ID NO: 346 - DNA, 55 bp, Artificial Sequence
  Synthetic Oligonucleotide
acactctttccctacacgacgctcttccgatctgggaaaacactctctctctgct

SEQ ID NO: 347 - DNA, 53 bp, Artificial Sequence
  Synthetic Oligonucleotide
acactctttccctacacgacgctcttccgatctggaggccacgacacacaata

SEQ ID NO: 348 - DNA, 54 bp, Artificial Sequence
  Synthetic Oligonucleotide
gtgactggagttcagacgtgtgctcttccgatctcacagggtggctcttcagtg

SEQ ID NO: 349 - DNA, 54 bp, Artificial Sequence
  Synthetic Oligonucleotide
gtgactggagttcagacgtgtgctcttccgatcttgcacatgtttccacagggt

SEQ ID NO: 350 - DNA, 54 bp, Artificial Sequence
  Synthetic Oligonucleotide
gtgactggagttcagacgtgtgctcttccgatctagtgtttccaggagcggttt

SEQ ID NO: 351 - DNA, 54 bp, Artificial Sequence
  Synthetic Oligonucleotide
gtgactggagttcagacgtgtgctcttccgatctaagcctcaggcacaactctg

SEQ ID NO: 352 - DNA, 53 bp, Artificial Sequence
  Synthetic Oligonucleotide
gtgactggagttcagacgtgtgctcttccgatcttaggggaggggcaaagaca

SEQ ID NO: 353 - DNA, 54 bp, Artificial Sequence
  Synthetic Oligonucleotide
gtgactggagttcagacgtgtgctcttccgatctgggaacagtggtatgctggt

SEQ ID NO: 354 - DNA, 55 bp, Artificial Sequence
  Synthetic Oligonucleotide
gtgactggagttcagacgtgtgctcttccgatctagtgtggacactgacaaggaa

SEQ ID NO: 355 - DNA, 54 bp, Artificial Sequence
  Synthetic Oligonucleotide
gtgactggagttcagacgtgtgctcttccgatcttcactgcctgggtgctttag

SEQ ID NO: 356 - DNA, 54 bp, Artificial Sequence
  Synthetic Oligonucleotide
gtgactggagttcagacgtgtgctcttccgatcttaccccagcctccagcttta

SEQ ID NO: 357 - DNA, 54 bp, Artificial Sequence
  Synthetic Oligonucleotide
gtgactggagttcagacgtgtgctcttccgatcttgactactggggagcgatga

SEQ ID NO: 358 - DNA, 56 bp, Artificial Sequence
  Synthetic Oligonucleotide
gtgactggagttcagacgtgtgctcttccgatctaggctgttatgcaggaaaggaa

SEQ ID NO: 359 - DNA, 54 bp, Artificial Sequence
  Synthetic Oligonucleotide
gtgactggagttcagacgtgtgctcttccgatctgcggttgaggtggatggaag

SEQ ID NO: 360 - DNA, 54 bp, Artificial Sequence
  Synthetic Oligonucleotide
gtgactggagttcagacgtgtgctcttccgatctggcagcatcccttacatcct

SEQ ID NO: 361 - DNA, 57 bp, Artificial Sequence
  Synthetic Oligonucleotide
gtgactggagttcagacgtgtgctcttccgatctagaaaaagcttccccagaaagga

SEQ ID NO: 362 - DNA, 54 bp, Artificial Sequence
  Synthetic Oligonucleotide
gtgactggagttcagacgtgtgctcttccgatctctgcaccaacctctacgtcc

SEQ ID NO: 363 - DNA, 54 bp, Artificial Sequence
  Synthetic Oligonucleotide
gtgactggagttcagacgtgtgctcttccgatctctggagagggcatagttggc

SEQ ID NO: 364 - DNA, 54 bp, Artificial Sequence
  Synthetic Oligonucleotide
gtgactggagttcagacgtgtgctcttccgatcttggaaggctctttgtgggtt

SEQ ID NO: 365 - DNA, 54 bp, Artificial Sequence
  Synthetic Oligonucleotide
gtgactggagttcagacgtgtgctcttccgatctttcctagcgggaactggaaa

SEQ ID NO: 366 - DNA, 54 bp, Artificial Sequence
  Synthetic Oligonucleotide
gtgactggagttcagacgtgtgctcttccgatctaggctaatggggtaggggat

SEQ ID NO: 367 - DNA, 54 bp, Artificial Sequence
  Synthetic Oligonucleotide
gtgactggagttcagacgtgtgctcttccgatcttgtccatgttggctgaggtg

SEQ ID NO: 368 - DNA, 54 bp, Artificial Sequence
  Synthetic Oligonucleotide
gtgactggagttcagacgtgtgctcttccgatctcaggccaaccttgacaactt

SEQ ID NO: 369 - DNA, 54 bp, Artificial Sequence
  Synthetic Oligonucleotide
gtgactggagttcagacgtgtgctcttccgatctagcaggccaaagatgtctcc

SEQ ID NO: 370 - DNA, 57 bp, Artificial Sequence
  Synthetic Oligonucleotide
gtgactggagttcagacgtgtgctcttccgatcttctgctcttgaggttatttgtcc

SEQ ID NO: 371 - DNA, 56 bp, Artificial Sequence
  Synthetic Oligonucleotide
gtgactggagttcagacgtgtgctcttccgatctgggaccaatttgctactcatgg

SEQ ID NO: 372 - DNA, 54 bp, Artificial Sequence
  Synthetic Oligonucleotide
gtgactggagttcagacgtgtgctcttccgatcttggaggctgtaaacgtcctg

SEQ ID NO: 373 - DNA, 59 bp, Artificial Sequence
  Synthetic Oligonucleotide
gtgactggagttcagacgtgtgctcttccgatcttgctatgatttgctgaattactcct

SEQ ID NO: 374 - DNA, 55 bp, Artificial Sequence
  Synthetic Oligonucleotide
gtgactggagttcagacgtgtgctcttccgatctgcaattttgcagaccaccatc

SEQ ID NO: 375 - DNA, 54 bp, Artificial Sequence
  Synthetic Oligonucleotide
gtgactggagttcagacgtgtgctcttccgatctggcagcttgcaaccttcttg

SEQ ID NO: 376 - DNA, 54 bp, Artificial Sequence
  Synthetic Oligonucleotide
gtgactggagttcagacgtgtgctcttccgatcttcatgagagtttccccaaca

SEQ ID NO: 377 - DNA, 58 bp, Artificial Sequence
  Synthetic Oligonucleotide
gtgactggagttcagacgtgtgctcttccgatctacttgagggggaaaaagtttctta

SEQ ID NO: 378 - DNA, 54 bp, Artificial Sequence
  Synthetic Oligonucleotide
gtgactggagttcagacgtgtgctcttccgatcttggtccctgtctgtcattgg

SEQ ID NO: 379 - DNA, 54 bp, Artificial Sequence
  Synthetic Oligonucleotide
gtgactggagttcagacgtgtgctcttccgatctaagcgagtgactgtctggga

SEQ ID NO: 380 - DNA, 54 bp, Artificial Sequence
  Synthetic Oligonucleotide
gtgactggagttcagacgtgtgctcttccgatctcatgggtgggacacgtagtt

SEQ ID NO: 381 - DNA, 55 bp, Artificial Sequence
  Synthetic Oligonucleotide
gtgactggagttcagacgtgtgctcttccgatctggctttcctggacaccctatc

SEQ ID NO: 382 - DNA, 53 bp, Artificial Sequence
  Synthetic Oligonucleotide
gtgactggagttcagacgtgtgctcttccgatctagagcgagggagcgatgta

SEQ ID NO: 383 - DNA, 55 bp, Artificial Sequence
  Synthetic Oligonucleotide
gtgactggagttcagacgtgtgctcttccgatctttgtggaccactgcttagtgc

SEQ ID NO: 384 - DNA, 53 bp, Artificial Sequence
  Synthetic Oligonucleotide
gtgactggagttcagacgtgtgctcttccgatctcaactaccctgaggccacc

SEQ ID NO: 385 - DNA, 54 bp, Artificial Sequence
  Synthetic Oligonucleotide
gtgactggagttcagacgtgtgctcttccgatctggtcagcactcctcagcttt

SEQ ID NO: 386 - DNA, 54 bp, Artificial Sequence
  Synthetic Oligonucleotide
gtgactggagttcagacgtgtgctcttccgatcttggaggatgcatgccacatt

SEQ ID NO: 387 - DNA, 54 bp, Artificial Sequence
  Synthetic Oligonucleotide
gtgactggagttcagacgtgtgctcttccgatctcccagcctctttgacccttc

SEQ ID NO: 388 - DNA, 53 bp, Artificial Sequence
  Synthetic Oligonucleotide
gtgactggagttcagacgtgtgctcttccgatctcccacaccaggctgtaagg

SEQ ID NO: 389 - DNA, 58 bp, Artificial Sequence
  Synthetic Oligonucleotide
gtgactggagttcagacgtgtgctcttccgatcttagatatatgggtgtgtctgtacg

SEQ ID NO: 390 - DNA, 54 bp, Artificial Sequence
  Synthetic Oligonucleotide
gtgactggagttcagacgtgtgctcttccgatctttccaaagtggctgaaccat

SEQ ID NO: 391 - DNA, 54 bp, Artificial Sequence
  Synthetic Oligonucleotide
gtgactggagttcagacgtgtgctcttccgatctcccacagggctgatgtttca

SEQ ID NO: 392 - DNA, 57 bp, Artificial Sequence
  Synthetic Oligonucleotide
gtgactggagttcagacgtgtgctcttccgatctttgtaatgcaacctctgtcatgc

SEQ ID NO: 393 - DNA, 54 bp, Artificial Sequence
  Synthetic Oligonucleotide
gtgactggagttcagacgtgtgctcttccgatctccagctccagcaatccatga

SEQ ID NO: 394 - DNA, 55 bp, Artificial Sequence
  Synthetic Oligonucleotide
gtgactggagttcagacgtgtgctcttccgatcttttgggaaagatagccctgga

SEQ ID NO: 395 - DNA, 54 bp, Artificial Sequence
  Synthetic Oligonucleotide
gtgactggagttcagacgtgtgctcttccgatctcaatgaaacagcggggaggt

SEQ ID NO: 396 - DNA, 54 bp, Artificial Sequence
  Synthetic Oligonucleotide
gtgactggagttcagacgtgtgctcttccgatctacaatcacgtgtccttcact

SEQ ID NO: 397 - DNA, 54 bp, Artificial Sequence
  Synthetic Oligonucleotide
gtgactggagttcagacgtgtgctcttccgatctcagatccctcctgggcaatg

SEQ ID NO: 398 - DNA, 54 bp, Artificial Sequence
  Synthetic Oligonucleotide
gtgactggagttcagacgtgtgctcttccgatctgtcaggaggcaaggaggaac

SEQ ID NO: 399 - DNA, 58 bp, Artificial Sequence
  Synthetic Oligonucleotide
gtgactggagttcagacgtgtgctcttccgatctacttccttccttttgagaccaagt

SEQ ID NO: 400 - DNA, 54 bp, Artificial Sequence
  Synthetic Oligonucleotide
gtgactggagttcagacgtgtgctcttccgatctgcggcagattcctggtgatt

SEQ ID NO: 401 - DNA, 54 bp, Artificial Sequence
  Synthetic Oligonucleotide
gtgactggagttcagacgtgtgctcttccgatctggtcaccatcagcacagtca

SEQ ID NO: 402 - DNA, 56 bp, Artificial Sequence
  Synthetic Oligonucleotide
caagcagaagacggcatacgagatatatcagtgtgactggagttcagacgtgtgct

SEQ ID NO: 403 - DNA, 56 bp, Artificial Sequence
  Synthetic Oligonucleotide
caagcagaagacggcatacgagattttcaccggtgactggagttcagacgtgtgct

SEQ ID NO: 404 - DNA, 56 bp, Artificial Sequence
  Synthetic Oligonucleotide
caagcagaagacggcatacgagatccactcatgtgactggagttcagacgtgtgct

SEQ ID NO: 405 - DNA, 56 bp, Artificial Sequence
  Synthetic Oligonucleotide
caagcagaagacggcatacgagattacgtacggtgactggagttcagacgtgtgct

SEQ ID NO: 406 - DNA, 56 bp, Artificial Sequence
  Synthetic Oligonucleotide
caagcagaagacggcatacgagatcgaaactcgtgactggagttcagacgtgtgct

SEQ ID NO: 407 - DNA, 56 bp, Artificial Sequence
  Synthetic Oligonucleotide
caagcagaagacggcatacgagatatcagtatgtgactggagttcagacgtgtgct

SEQ ID NO: 408 - DNA, 57 bp, Artificial Sequence
  Synthetic Oligonucleotide
aatgatacggcgaccaccgagatctacacattactcgacactctttccctacacgac

SEQ ID NO: 409 - DNA, 57 bp, Artificial Sequence
  Synthetic Oligonucleotide
aatgatacggcgaccaccgagatctacactccggagaacactctttccctacacgac

SEQ ID NO: 410 - DNA, 57 bp, Artificial Sequence
  Synthetic Oligonucleotide
aatgatacggcgaccaccgagatctacaccgctcattacactctttccctacacgac